European Patent Application EP 4 112 089 A1, published January 4, 2023. Title: Material for preventing leakage of digestive liquid from digestive organ and material for protecting organ from digestion by digestive liquid. Applicant: Menicon Co., Ltd. Osaka University. The sequence listing filed with the application follows.

SEQUENCE LISTING (18 sequences)

SEQ ID NO: 1 - protein, 13 aa, Artificial Sequence
  self-assembling peptide
RLDLRLALRLDLR

SEQ ID NO: 2 - protein, 13 aa, Artificial Sequence
  self-assembling peptide
RLDLRLSLRLDLR

SEQ ID NO: 3 - protein, 13 aa, Artificial Sequence
  self-assembling peptide
RLALRLDLRLDLR

SEQ ID NO: 4 - protein, 13 aa, Artificial Sequence
  self-assembling peptide
KRLDLNLRLDLRK

SEQ ID NO: 5 - protein, 13 aa, Artificial Sequence
  self-assembling peptide
RLDLRLLLRLDLR

SEQ ID NO: 6 - protein, 13 aa, Artificial Sequence
  self-assembling peptide
RADLRLALRLDLR

SEQ ID NO: 7 - protein, 13 aa, Artificial Sequence
  self-assembling peptide
RLDLRLALRLDAR

SEQ ID NO: 8 - protein, 13 aa, Artificial Sequence
  self-assembling peptide
RADLRLLLRLDLR

SEQ ID NO: 9 - protein, 13 aa, Artificial Sequence
  self-assembling peptide
RADLRLLLRLDAR

SEQ ID NO: 10 - protein, 13 aa, Artificial Sequence
  self-assembling peptide
RLDLRALLRLDLR

SEQ ID NO: 11 - protein, 13 aa, Artificial Sequence
  self-assembling peptide
RLDLRLLARLDLR

SEQ ID NO: 12 - protein, 12 aa, Artificial Sequence
  self-assembling peptide
RLNLRLDLRLNL

SEQ ID NO: 13 - protein, 16 aa, Artificial Sequence
  self-assembling peptide
RAQARAQARAQARAQA

SEQ ID NO: 14 - protein, 16 aa, Artificial Sequence
  self-assembling peptide
SAEASAEASAEAKAEA

SEQ ID NO: 15 - protein, 16 aa, Artificial Sequence
  self-assembling peptide
RADARADARADARADA

SEQ ID NO: 16 - protein, 16 aa, Artificial Sequence
  self-assembling peptide
RASARASARASARASA

SEQ ID NO: 17 - protein, 16 aa, Artificial Sequence
  self-assembling peptide
RASARASARASARADA

SEQ ID NO: 18 - protein, 16 aa, Artificial Sequence
  self-assembling peptide
RASARADARADARADA